European Patent Specification EP 3 638 284 B1, published August 30, 2023. Title: Cyclic Peptides. Applicant: Virometix AG Universität Zürich. The sequence listing filed with the application follows.

SEQUENCE LISTING (57 sequences)

SEQ ID NO: 1 - protein, 30 aa, Artificial Sequence
  Synthetic sequence
  MISC_FEATURE (1)..(3): Amino acid Xaa
  MISC_FEATURE (5)..(7): Amino acid Xaa
  MISC_FEATURE (9)..(11): Amino acid Xaa
  MISC_FEATURE (22)..(24): Amino acid Xaa
  MISC_FEATURE (26)..(30): Amino acid Xaa
XXXCXXXCXXXPITNDQKKLCXXXCXXXXX

SEQ ID NO: 2 - protein, 30 aa, Artificial Sequence
  Synthetic sequence
  MOD_RES (11)..(11): Nle
  MOD_RES (24)..(24): Dbu
  MISC_FEATURE (30)..(30): D-alanine
NSECLSLCNDXPITNDQKKLCSNXCQSVRX

SEQ ID NO: 3 - protein, 30 aa, Artificial Sequence
  Synthetic sequence
  MOD_RES (11)..(11): Nle
  MISC_FEATURE (30)..(30): D-alanine
NSECLSLCNDXPITNDQKKLCSNKCQSVRX

SEQ ID NO: 4 - protein, 30 aa, Artificial Sequence
  Synthetic sequence
  MOD_RES (12)..(12): Nle
  MISC_FEATURE (30)..(30): D-alanine
RLSECLSLCNDXPITNDQKKLCSNNCLKSX

SEQ ID NO: 5 - protein, 40 aa, Artificial Sequence
  Synthetic sequence
  MISC_FEATURE (40)..(40): D-alanine
PVSTYMLTNSECLSLCNDMPITNDQKKLCSNNCQIVRQQX

SEQ ID NO: 6 - protein, 20 aa, Artificial Sequence
  T helper cell epitope
IEKKIAKMEKASSVFNVVNS

SEQ ID NO: 7 - protein, 10 aa, Artificial Sequence
  FSL-1
  BINDING (1)..(1): S-(2,3-bispalmitoyloxypropyl)
CGDPKHPKSF

SEQ ID NO: 8 - protein, 10 aa, Artificial Sequence
  FSL-2
  BINDING (1)..(1): S-(2,3-bispalmitoyloxypropyl)
CGDPKHPKSR

SEQ ID NO: 9 - protein, 10 aa, Artificial Sequence
  FSL-3
  BINDING (1)..(1): S-(2,3-bisstearyloxypropyl)
CGDPKHPKSF

SEQ ID NO: 10 - protein, 14 aa, Artificial Sequence
  MALP-2
  BINDING (1)..(1): S-(2,3-bispalmitoyloxypropyl)
CGNNDESNISFKEK

SEQ ID NO: 11 - protein, 5 aa, Artificial Sequence
  C-terminal sequence
  MISC_FEATURE (5)..(5): D-alanine
KKKCX

SEQ ID NO: 12 - protein, 7 aa, Artificial Sequence
  heptad motif
IEKKIEA

SEQ ID NO: 13 - protein, 7 aa, Artificial Sequence
  heptad motif
IEKKIES

SEQ ID NO: 14 - protein, 30 aa, Artificial Sequence
  Synthetic
  BINDING (1)..(1): Maleimido moiety
  MOD_RES (11)..(11): Nle
  MOD_RES (21)..(21): Nle
  MISC_FEATURE (30)..(30): D-alanine
  MOD_RES (30)..(30): AMIDATION
NSELLSLINDXPITNDQKKLXSNNVQSVRX

SEQ ID NO: 15 - protein, 30 aa, Artificial Sequence
  Synthetic
  BINDING (1)..(1): AoAc miety incl. a  1-amino-3,6,9,12,15,18-hexaoxaheneicosan-21- oic amide linker
  MOD_RES (11)..(11): Nle
  MOD_RES (24)..(24): Dbu
  MISC_FEATURE (30)..(30): D-alanine
  MOD_RES (30)..(30): AMIDATION
NSELLSLCNDXPITNDQKKLCSNXVQSVRX

SEQ ID NO: 16 - protein, 30 aa, Artificial Sequence; identical to SEQ ID NO: 2
  Synthetic
  BINDING (1)..(1): AoAc moiety incl. 1-amino-3,6,9,12,15,18-hexaoxaheneicosan-21-oic amide linker
  MOD_RES (11)..(11): Nle
  MOD_RES (24)..(24): Dbu
  MISC_FEATURE (30)..(30): D-alanine
  MOD_RES (30)..(30): AMIDATION

SEQ ID NO: 17 - protein, 30 aa, Artificial Sequence; identical to SEQ ID NO: 2
  Synthetic
  BINDING (1)..(1): AoAc moiety
  MOD_RES (11)..(11): Nle
  MOD_RES (24)..(24): Dbu
  MISC_FEATURE (30)..(30): D-alanine
  MOD_RES (30)..(30): AMIDATION

SEQ ID NO: 18 - protein, 30 aa, Artificial Sequence; identical to SEQ ID NO: 3
  Synthetic
  BINDING (1)..(1): Ac moiety
  MOD_RES (11)..(11): Nle
  BINDING (24)..(24): AOAc moiety
  MISC_FEATURE (30)..(30): D-alanine
  MOD_RES (30)..(30): AMIDATION

SEQ ID NO: 19 - protein, 30 aa, Artificial Sequence; identical to SEQ ID NO: 4
  Synthetic
  BINDING (1)..(1): AOAc
  MOD_RES (12)..(12): Nle
  MISC_FEATURE (30)..(30): D-alanine
  MOD_RES (30)..(30): AMIDATION

SEQ ID NO: 20 - protein, 40 aa, Artificial Sequence; identical to SEQ ID NO: 5
  Synthetic
  BINDING (1)..(1): AOAc
  MISC_FEATURE (40)..(40): D-alanine
  MOD_RES (40)..(40): AMIDATION

SEQ ID NO: 21 - protein, 30 aa, Artificial Sequence
  Synthetic
  MOD_RES (11)..(11): Nle
  MISC_FEATURE (30)..(30): D-alanine
NSECLSLCNDXPITNDQKKLCSNNCQSVRX

SEQ ID NO: 22 - protein, 30 aa, Artificial Sequence
  Synthetic
  MOD_RES (11)..(11): Nle
  MISC_FEATURE (30)..(30): D-alanine
NSECLSLCNDXPITNDQKKLCSNDCQSVRX

SEQ ID NO: 23 - protein, 30 aa, Artificial Sequence; identical to SEQ ID NO: 2
  Synthetic
  MOD_RES (11)..(11): Nle
  MOD_RES (24)..(24): Orn
  MISC_FEATURE (30)..(30): D-alanine

SEQ ID NO: 24 - protein, 30 aa, Artificial Sequence
  Synthetic
  MOD_RES (12)..(12): Nle
  MISC_FEATURE (30)..(30): D-alanine
RLSECLSLCNDXPITNDQKKLCSNKCLKSX

SEQ ID NO: 25 - protein, 30 aa, Artificial Sequence
  Synthetic
  MOD_RES (12)..(12): Nle
  MOD_RES (25)..(25): Dbu
  MISC_FEATURE (30)..(30): D-alanine
RLSECLSLCNDXPITNDQKKLCSNXCLKSX

SEQ ID NO: 26 - protein, 40 aa, Artificial Sequence
  Synthetic
  MISC_FEATURE (40)..(40): D-alanine
PVSTYMLTNSECLSLCNDMPITNDQKKLCSNKCQIVRQQX

SEQ ID NO: 27 - protein, 40 aa, Artificial Sequence
  Synthetic
  MOD_RES (32)..(32): Dbu
  MISC_FEATURE (40)..(40): D-alanine
PVSTYMLTNSECLSLCNDMPITNDQKKLCSNXCQIVRQQX

SEQ ID NO: 28 - protein, 30 aa, Artificial Sequence
  Synthetic
  MOD_RES (12)..(12): Nle
  MISC_FEATURE (30)..(30): D-alanine
RLSECLSLCNDXPITNDQKKLCSNDCLKSX

SEQ ID NO: 29 - protein, 30 aa, Artificial Sequence; identical to SEQ ID NO: 25
  Synthetic
  MOD_RES (12)..(12): Nle
  MOD_RES (25)..(25): Orn
  MISC_FEATURE (30)..(30): D-alanine

SEQ ID NO: 30 - protein, 40 aa, Artificial Sequence
  Synthetic
  MISC_FEATURE (40)..(40): D-alanine
PVSTYMLTNSECLSLCNDMPITNDQKKLCSNDCQIVRQQX

SEQ ID NO: 31 - protein, 40 aa, Artificial Sequence; identical to SEQ ID NO: 27
  Synthetic
  MOD_RES (32)..(32): Orn
  MISC_FEATURE (40)..(40): D-alanine

SEQ ID NO: 32 - protein, 40 aa, Artificial Sequence
  Synthetic
  MOD_RES (19)..(19): Nle
  MISC_FEATURE (40)..(40): D-alanine
PVSTYMLTNSECLSLCNDXPITNDQKKLCSNNCQIVRQQX

SEQ ID NO: 33 - protein, 40 aa, Artificial Sequence
  Synthetic
  MOD_RES (19)..(19): Nle
  MISC_FEATURE (40)..(40): X-alanine
PVSTYMLTNSECLSLCNDXPITNDQKKLCSNKCQIVRQQX

SEQ ID NO: 34 - protein, 40 aa, Artificial Sequence
  Synthetic
  MOD_RES (19)..(19): Nle
  MOD_RES (32)..(32): Dbu
  MISC_FEATURE (40)..(40): D-alanine
PVSTYMLTNSECLSLCNDXPITNDQKKLCSNXCQIVRQQX

SEQ ID NO: 35 - protein, 40 aa, Artificial Sequence
  Synthetic
  MOD_RES (19)..(19): Nle
  MISC_FEATURE (40)..(40): D-alanine
PVSTYMLTNSECLSLCNDXPITNDQKKLCSNDCQIVRQQX

SEQ ID NO: 36 - protein, 40 aa, Artificial Sequence; identical to SEQ ID NO: 34
  Synthetic
  MOD_RES (19)..(19): Nle
  MOD_RES (32)..(32): Dbu
  MOD_RES (32)..(32): orn
  MISC_FEATURE (40)..(40): D-alanine

SEQ ID NO: 37 - protein, 30 aa, Artificial Sequence; identical to SEQ ID NO: 14
  Synthetic
  MOD_RES (11)..(11): Nle
  MOD_RES (21)..(21): Nle
  MISC_FEATURE (30)..(30): D-alanine

SEQ ID NO: 38 - protein, 30 aa, Artificial Sequence; identical to SEQ ID NO: 15
  Synthetic
  MOD_RES (11)..(11): Nle
  MOD_RES (24)..(24): Dbu
  MISC_FEATURE (30)..(30): D-alanine

SEQ ID NO: 39 - protein, 30 aa, Artificial Sequence
  Synthetic
  MOD_RES (11)..(11): Nle
  MOD_RES (24)..(24): Dbu
  MISC_FEATURE (30)..(30): D-alanine
NSECLSLCNDXPITNDQKKLCSSXCQSVRX

SEQ ID NO: 40 - protein, 30 aa, Artificial Sequence
  Synthetic
  MOD_RES (11)..(11): Nle
  MISC_FEATURE (30)..(30): D-alanine
NSECLSLCNDXPITNDQKKLCSSNCQSVRX

SEQ ID NO: 41 - protein, 30 aa, Artificial Sequence
  Synthetic
  MOD_RES (11)..(11): Nle
  MISC_FEATURE (30)..(30): D-alanine
NSECLSLCNDXPITNDQKKLCSSQCQSVRX

SEQ ID NO: 42 - protein, 30 aa, Artificial Sequence
  Synthetic
  MOD_RES (11)..(11): Nle
  MOD_RES (30)..(30): AMIDATION
  MISC_FEATURE (30)..(30): D-alanine
NSECLSLCNDXPITNDQKKLCSSSCQSVRX

SEQ ID NO: 43 - protein, 30 aa, Artificial Sequence
  Synthetic
  MOD_RES (11)..(11): Nle
  MOD_RES (24)..(24): Dbu
  MISC_FEATURE (30)..(30): D-alanine
QSECLSLCNDXPITNDQKKLCSNXCQSVRX

SEQ ID NO: 44 - protein, 30 aa, Artificial Sequence
  Synthetic
  MOD_RES (11)..(11): Nle
  MOD_RES (24)..(24): Dbu
  MISC_FEATURE (30)..(30): D-alanine
QSECLSLCNDXPITNDQKKLCSSXCQSVRX

SEQ ID NO: 45 - protein, 30 aa, Artificial Sequence
  Synthetic
  MOD_RES (11)..(11): Nle
  MISC_FEATURE (30)..(30): D-alanine
QSECLSLCNDXPITNDQKKLCSSNCQSVRX

SEQ ID NO: 46 - protein, 30 aa, Artificial Sequence
  Synthetic
  MOD_RES (11)..(11): Nle
  MISC_FEATURE (30)..(30): D-alanine
QSECLSLCNDXPITNDQKKLCSSQCQSVRX

SEQ ID NO: 47 - protein, 30 aa, Artificial Sequence
  Synthetic
  MOD_RES (11)..(11): Nle
  MISC_FEATURE (30)..(30): D-alanine
QSECLSLCNDXPITNDQKKLCSSSCQSVRX

SEQ ID NO: 48 - protein, 30 aa, Artificial Sequence
  Synthetic
  MOD_RES (11)..(11): Nle
  MOD_RES (24)..(24): Dbu
  MISC_FEATURE (30)..(30): D-alanine
SSECLSLCNDXPITNDQKKLCSNXCQSVRX

SEQ ID NO: 49 - protein, 30 aa, Artificial Sequence
  Synthetic
  MOD_RES (11)..(11): Nle
  MOD_RES (24)..(24): Dbu
  MISC_FEATURE (30)..(30): D-alanine
SSECLSLCNDXPITNDQKKLCSSXCQSVRX

SEQ ID NO: 50 - protein, 30 aa, Artificial Sequence
  Synthetic
  MOD_RES (11)..(11): Nle
  MISC_FEATURE (30)..(30): D-alanine
SSECLSLCNDXPITNDQKKLCSSNCQSVRX

SEQ ID NO: 51 - protein, 30 aa, Artificial Sequence
  Synthetic
  MOD_RES (11)..(11): Nle
  MISC_FEATURE (30)..(30): D-alanine
SSECLSLCNDXPITNDQKKLCSSQCQSVRX

SEQ ID NO: 52 - protein, 30 aa, Artificial Sequence
  Synthetic
  MOD_RES (11)..(11): Nle
  MISC_FEATURE (30)..(30): D-alanine
SSECLSLCNDXPITNDQKKLCSSSCQSVRX

SEQ ID NO: 53 - protein, 30 aa, Artificial Sequence
  Synthetic
  MOD_RES (11)..(11): Nle
  MOD_RES (24)..(24): Dbu
  MISC_FEATURE (30)..(30): D-alanine
GSECLSLCNDXPITNDQKKLCSNXCQSVRX

SEQ ID NO: 54 - protein, 30 aa, Artificial Sequence
  Synthetic
  MOD_RES (11)..(11): Nle
  MOD_RES (24)..(24): Dbu
  MISC_FEATURE (30)..(30): D-alanine
GSECLSLCNDXPITNDQKKLCSSXCQSVRX

SEQ ID NO: 55 - protein, 30 aa, Artificial Sequence
  Synthetic
  MOD_RES (11)..(11): Nle
  MISC_FEATURE (30)..(30): D-alanine
GSECLSLCNDXPITNDQKKLCSSNCQSVRX

SEQ ID NO: 56 - protein, 30 aa, Artificial Sequence
  Synthetic
  MOD_RES (11)..(11): Nle
  MISC_FEATURE (30)..(30): D-alanine
GSECLSLCNDXPITNDQKKLCSSQCQSVRX

SEQ ID NO: 57 - protein, 30 aa, Artificial Sequence
  Synthetic
  MOD_RES (11)..(11): Nle
  MISC_FEATURE (30)..(30): D-alanine
GSECLSLCNDXPITNDQKKLCSSSCQSVRX